European Patent Application EP 4 389 138 A1, published June 26, 2024. Title: Dosage Regimen for Interleukin-22 Derivatives. Applicant: CytoKi Pharma ApS. Application EP. The sequence listing filed with the application follows.

SEQUENCE LISTING (34 sequences)

SEQ ID NO: 1 - protein, 146 aa, Homo sapiens
APISSHCRLDKSNFQQPYITNRTFMLAKEASLADNNTDVRLIGEKLFHGVSMSERCYLMKQVLNFTLEEVLFPQSDRFQPYMQEVVPFLARLSNRLSTCHIEGDDLHIQRNVQKLKDTVKKLGESGEIKAIGELDLLFMSLRNACI

SEQ ID NO: 2 - protein, 5 aa, synthetic construct
  REGION 1..5: note = n-mer that can be inserted in SEQ ID NO. 1 (to create an experimentally altered version of SEQ ID NO. 1)
RVQFQ

SEQ ID NO: 3 - protein, 5 aa, synthetic construct
  REGION 1..5: note = n-mer that can be inserted in SEQ ID NO. 1 (to create an experimentally altered version of SEQ ID NO. 1)
CVEIP

SEQ ID NO: 4 - protein, 7 aa, synthetic construct
  REGION 1..7: note = n-mer that can be inserted in SEQ ID NO. 1 (to create an experimentally altered version of SEQ ID NO. 1)
GSGSGSC

SEQ ID NO: 5 - protein, 8 aa, synthetic construct
  REGION 1..8: note = n-mer that can be inserted in SEQ ID NO. 1 (to create an experimentally altered version of SEQ ID NO. 1)
IEALTPHS

SEQ ID NO: 6 - protein, 8 aa, synthetic construct
  REGION 1..8: note = n-mer that can be inserted in SEQ ID NO. 1 (to create an experimentally altered version of SEQ ID NO. 1)
YGQRQWKN

SEQ ID NO: 7 - protein, 9 aa, synthetic construct
  REGION 1..9: note = n-mer that can be inserted in SEQ ID NO. 1 (to create an experimentally altered version of SEQ ID NO. 1)
VFIINNSLE

SEQ ID NO: 8 - protein, 44 aa, synthetic construct
  REGION 1..44: note = n-mer that can be inserted in SEQ ID NO. 1 (to create an experimentally altered version of SEQ ID NO. 1)
RAASAGSYSEWSMTPRFTPWWETKIDPPVMNITQVNGSLLVILH

SEQ ID NO: 9 - protein, 5 aa, synthetic construct
  REGION 1..5: note = n-mer that can be added as an N-terminal peptide on SEQ ID NO. 1 (to create an experimentally altered version of SEQ ID NO. 1)
AEPEE

SEQ ID NO: 10 - protein, 7 aa, synthetic construct
  REGION 1..7: note = n-mer that can be added as an N-terminal peptide on SEQ ID NO. 1 (to create an experimentally altered version of SEQ ID NO. 1)
GPAEPEE

SEQ ID NO: 11 - protein, 8 aa, synthetic construct
  REGION 1..8: note = n-mer that can be added as an N-terminal peptide on SEQ ID NO. 1 (to create an experimentally altered version of SEQ ID NO. 1)
GPACEPEE

SEQ ID NO: 12 - protein, 12 aa, synthetic construct
  REGION 1..12: note = n-mer that can be added as an N-terminal peptide on SEQ ID NO. 1 (to create an experimentally altered version of SEQ ID NO. 1)
GSGSGSGSGSGS

SEQ ID NO: 13 - protein, 13 aa, synthetic construct
  REGION 1..13: note = n-mer that can be added as an N-terminal peptide on SEQ ID NO. 1 (to create an experimentally altered version of SEQ ID NO. 1)
GGSSGSGSEVLFQ

SEQ ID NO: 14 - protein, 14 aa, synthetic construct
  REGION 1..14: note = n-mer that can be added as an N-terminal peptide on SEQ ID NO. 1 (to create an experimentally altered version of SEQ ID NO. 1)
GPGSGSGSGSGSGS

SEQ ID NO: 15 - protein, 14 aa, synthetic construct
  REGION 1..14: note = n-mer that can be added as an N-terminal peptide on SEQ ID NO. 1 (to create an experimentally altered version of SEQ ID NO. 1)
GGSSGSGSEVLFQG

SEQ ID NO: 16 - protein, 15 aa, synthetic construct
  REGION 1..15: note = n-mer that can be added as an N-terminal peptide on SEQ ID NO. 1 (to create an experimentally altered version of SEQ ID NO. 1)
GPGSGSGSCGSGSGS

SEQ ID NO: 17 - protein, 16 aa, synthetic construct
  REGION 1..16: note = n-mer that can be added as an N-terminal peptide on SEQ ID NO. 1 (to create an experimentally altered version of SEQ ID NO. 1)
GGSSGSGSEVLFQGPG

SEQ ID NO: 18 - protein, 20 aa, synthetic construct
  REGION 1..20: note = n-mer that can be added as an N-terminal peptide on SEQ ID NO. 1 (to create an experimentally altered version of SEQ ID NO. 1)
GGSSGSGSEVLFQGPAEPEE

SEQ ID NO: 19 - protein, 21 aa, synthetic construct
  REGION 1..21: note = n-mer that can be added as an N-terminal peptide on SEQ ID NO. 1 (to create an experimentally altered version of SEQ ID NO. 1)
GGSSGSGSEVLFQGPACEPEE

SEQ ID NO: 20 - protein, 27 aa, synthetic construct
  REGION 1..27: note = n-mer that can be added as an N-terminal peptide on SEQ ID NO. 1 (to create an experimentally altered version of SEQ ID NO. 1)
GGSSGSGSEVLFQGPGSGSGSGSGSGS

SEQ ID NO: 21 - protein, 28 aa, synthetic construct
  REGION 1..28: note = n-mer that can be added as an N-terminal peptide on SEQ ID NO. 1 (to create an experimentally altered version of SEQ ID NO. 1)
GGSSGSGSEVLFQGPGSGSGSCGSGSGS

SEQ ID NO: 22 - protein, 7 aa, synthetic construct
  REGION 1..7: note = n-mer that can be added as a C-terminal peptide on SEQ ID NO. 1 (to create an experimentally altered version of SEQ ID NO. 1)
GSGSGSC

SEQ ID NO: 23 - protein, 149 aa, synthetic construct
  REGION 1..149: note = Experimentally altered version of SEQ ID NO. 1
GPGCPISSHCRLDKSNFQQPYITNRTFMLAKEASLADNNTDVRLIGEKLFHGVSMSERCYLMKQVLNFTLEEVLFPQSDRFQPYMQEVVPFLARLSNRLSTCHIEGDDLHIQRNVQKLKDTVKKLGESGEIKAIGELDLLFMSLRNACI

SEQ ID NO: 24 - protein, 161 aa, synthetic construct
  REGION 1..161: note = Experimentally altered version of SEQ ID NO. 1
GPGSGSGSCGSGSGSAPISSHCRLDKSNFQQPYITNRTFMLAKEASLADNNTDVRLIGEKLFHGVSMSERCYLMKQVLNFTLEEVLFPQSDRFQPYMQEVVPFLARLSNRLSTCHIEGDDLHIQRNVQKLKDTVKKLGESGEIKAIGELDLLFMSLRNACI

SEQ ID NO: 25 - protein, 149 aa, synthetic construct
  REGION 1..149: note = Experimentally altered version of SEQ ID NO. 1
GPGCPISSHCRLDKSNFQQPYITNRTFMLAKEASLADQNTDVRLIGEKLFHGVSMSERCYLMKQVLQFTLEEVLFPQSDRFQPYMQEVVPFLARLSNRLSTCHIEGDDLHIQRNVQKLKDTVKKLGESGEIKAIGELDLLFMSLRNACI

SEQ ID NO: 26 - protein, 146 aa, synthetic construct
  REGION 1..146: note = Experimentally altered version of SEQ ID NO. 1
CPISSHCRLDKSNFQQPYITNRTFMLAKEASLADQNTDVRLIGEKLFHGVSMSERCYLMKQVLQFTLEEVLFPQSDRFQPYMQEVVPFLARLSNRLSTCHIEGDDLHIQRNVQKLKDTVKKLGESGEIKAIGELDLLFMSLRNACI

SEQ ID NO: 27 - protein, 147 aa, synthetic construct
  REGION 1..147: note = Experimentally altered version of SEQ ID NO. 1
GAPISSCCRLDKSNFQQPYITNRTFMLAKEASLADQNTDVRLIGEKLFHGVSMSERCYLMKQVLQFTLEEVLFPQSDRFQPYMQEVVPFLARLSNRLSTCHIEGDDLHIQRNVQKLKDTVKKLGESGEIKAIGELDLLFMSLRNACI

SEQ ID NO: 28 - protein, 146 aa, synthetic construct
  REGION 1..146: note = Experimentally altered version of SEQ ID NO. 1
APISSHCRLDKSNFQQPYITNRTFMLAKEASLCDQNTDVRLIGEKLFHGVSMSERCYLMKQVLQFTLEEVLFPQSDRFQPYMQEVVPFLARLSNRLSTCHIEGDDLHIQRNVQKLKDTVKKLGESGEIKAIGELDLLFMSLRNACI

SEQ ID NO: 29 - protein, 146 aa, synthetic construct
  REGION 1..146: note = Experimentally altered version of SEQ ID NO. 1
APISSHCRLDKSNFQQPYITNRTFMLAKEASLADQNTDVRLIGEKLFHGVSMSERCYLMKQVLQFTLEEVLFPQSDRFQPYMQEVVPFLARLSNRLSTCHIEGDDCHIQRNVQKLKDTVKKLGESGEIKAIGELDLLFMSLRNACI

SEQ ID NO: 30 - protein, 146 aa, synthetic construct
  REGION 1..146: note = Experimentally altered version of SEQ ID NO. 1
APISSHCRLDKSNFQQPYITNRTFMLAKEASLADQNTDVRLIGEKLFHGVSMSERCYLMKQVLQFTLEEVLFPQSDRFQPYMQEVVPFLARLSNCLSTCHIEGDDLHIQRNVQKLKDTVKKLGESGEIKAIGELDLLFMSLRNACI

SEQ ID NO: 31 - protein, 146 aa, synthetic construct
  REGION 1..146: note = Experimentally altered version of SEQ ID NO. 1
APISSHCRLDKSNFQQPYITNRTFMLAKEASLADNNTDVRLIGEKLFHGVSMSERCYLMKQVLNFTLEEVLFPQSDRFQPYMQEVVPFLARLSNRLSTCHIEGDDCHIQRNVQKLKDTVKKLGESGEIKAIGELDLLFMSLRNACI

SEQ ID NO: 32 - protein, 146 aa, synthetic construct
  REGION 1..146: note = Experimentally altered version of SEQ ID NO. 1
APISSHCRLDKSNFQQPYITNRTFMLAKEASLADNNTDVRLIGEKLFHGVSMSERCYLMKQVLNFTLEEVLFPQSDRFQPYMQEVVPFLARLSNCLSTCHIEGDDLHIQRNVQKLKDTVKKLGESGEIKAIGELDLLFMSLRNACI

SEQ ID NO: 33 - protein, 19 aa, synthetic construct
  REGION 1..19: note = His-tag
HHHHHHGGSSGSGSEVLFQ

SEQ ID NO: 34 - protein, 7 aa, synthetic construct
  REGION 1..7: note = Consensus sequence for native cut site in protease-cleavable TEV linker
ENLYFQS